European Patent Specification EP 3 849 996 B1, published April 22, 2026. Title: EPITOPE TAGS RECOGNIZED BY SPECIFIC BINDERS. Applicant: NanoTag Biotechnologies GmbH. The sequence listing filed with the application follows.

SEQUENCE LISTING (199 sequences)

SEQ ID NO: 1 - protein, 13 aa, Artificial Sequence
  synthetic peptide
  misc_feature (1)..(9): Xaa can be any naturally occurring amino acid
  misc_feature (12)..(13): Xaa can be any naturally occurring amino acid
XXXXXXXXXRLXX

SEQ ID NO: 2 - protein, 13 aa, Artificial Sequence
  synthetic peptide
  MISC_FEATURE (1)..(1): Xaa is G or S or P or T
  MISC_FEATURE (2)..(2): Xaa is R or G or P
  MISC_FEATURE (5)..(5): Xaa is E or Q
  MISC_FEATURE (7)..(7): Xaa is L or I
  MISC_FEATURE (12)..(12): Xaa is S or T or P or A or D or E
  MISC_FEATURE (13)..(13): Xaa is P or A or S or A or D or E or no amino acid
XXLEXEXRRRLXX

SEQ ID NO: 3 - protein, 13 aa, Artificial Sequence
  synthetic peptide
  MISC_FEATURE (1)..(1): Xaa is S or T
  MISC_FEATURE (2)..(2): Xaa is R or G
  MISC_FEATURE (5)..(5): Xaa is E or Q
  MISC_FEATURE (12)..(12): Xaa is T or D or E
  MISC_FEATURE (13)..(13): Xaa is A or D or E or no amino acid
XXLEXELRRRLXX

SEQ ID NO: 4 - protein, 13 aa, Artificial Sequence
  synthetic peptide
SRLEEELRRRLTE

SEQ ID NO: 5 - protein, 16 aa, Artificial Sequence
  synthetic peptide
MPSRLEEELRRRLTEP

SEQ ID NO: 6 - protein, 15 aa, Artificial Sequence
  synthetic peptide
PSRLEEELRRRLTEP

SEQ ID NO: 7 - protein, 14 aa, Artificial Sequence
  synthetic peptide
PSRLEEELRRRLTE

SEQ ID NO: 8 - protein, 15 aa, Artificial Sequence
  synthetic peptide
GRSRLEEELRRRLTA

SEQ ID NO: 9 - protein, 16 aa, Artificial Sequence
  synthetic peptide
PGSRLEEELRRRLTAP

SEQ ID NO: 10 - protein, 16 aa, Artificial Sequence
  synthetic peptide
PSTRLEEELRRRLTAP

SEQ ID NO: 11 - protein, 16 aa, Artificial Sequence
  synthetic peptide
SPSRLEEELRRRLTAP

SEQ ID NO: 12 - protein, 16 aa, Artificial Sequence
  synthetic peptide
  MISC_FEATURE (1)..(1): Xaa is G or S or T or P
  MISC_FEATURE (2)..(2): Xaa is R or G or A or E or P
  MISC_FEATURE (3)..(3): Xaa is L or V
  MISC_FEATURE (4)..(4): Xaa is E or Q
  MISC_FEATURE (5)..(5): Xaa is E or Q
  MISC_FEATURE (6)..(6): Xaa is E or Q
  MISC_FEATURE (7)..(7): Xaa is L or I or V
  MISC_FEATURE (8)..(8): Xaa is R or A or Q or E
  MISC_FEATURE (9)..(9): Xaa is R or A or Q or E
  MISC_FEATURE (12)..(12): Xaa is S or T  or D or E or P or A or no amino acid
  MISC_FEATURE (13)..(13): Xaa is E or K or P or S or A or D or no amino acid
SPSRLEEELRRRLDAP

SEQ ID NO: 13 - protein, 16 aa, Artificial Sequence
  synthetic peptide
SPSRLEEELRRRLEAP

SEQ ID NO: 14 - protein, 16 aa, Artificial Sequence
  synthetic peptide
SPSRLEEELRRRLTDP

SEQ ID NO: 15 - protein, 16 aa, Artificial Sequence
  synthetic peptide
SPSRLEEELRRRLTEP

SEQ ID NO: 16 - protein, 17 aa, Artificial Sequence
  synthetic peptide
SPSRLEEELRRRLTADP

SEQ ID NO: 17 - protein, 16 aa, Artificial Sequence
  synthetic peptide
SPSGLEEELRRRLTEP

SEQ ID NO: 18 - protein, 14 aa, Artificial Sequence
  synthetic peptide
GPSRLEEELRRRLT

SEQ ID NO: 19 - protein, 15 aa, Artificial Sequence
  synthetic peptide
GPSRLEEELRRRLTA

SEQ ID NO: 20 - protein, 16 aa, Artificial Sequence
  synthetic peptide
GPSRLEEELRRRLTAA

SEQ ID NO: 21 - protein, 17 aa, Artificial Sequence
  synthetic peptide
GPSRLEEELRRRLTAAS

SEQ ID NO: 22 - protein, 16 aa, Artificial Sequence
  synthetic peptide
SPSGLEQELRRRLTAP

SEQ ID NO: 23 - protein, 16 aa, Artificial Sequence
  synthetic peptide
SPSGLEQELRRRLDAP

SEQ ID NO: 24 - protein, 16 aa, Artificial Sequence
  synthetic peptide
SPSGLEQELRRRLEAP

SEQ ID NO: 25 - protein, 16 aa, Artificial Sequence
  synthetic peptide
SPSGLEQELRRRLTEP

SEQ ID NO: 26 - protein, 16 aa, Artificial Sequence
  synthetic peptide
GPSRLEEELRRRLTAP

SEQ ID NO: 27 - protein, 16 aa, Artificial Sequence
  synthetic peptide
GPSRLEEELRRRLTEP

SEQ ID NO: 28 - protein, 15 aa, Artificial Sequence
  synthetic peptide
GPSRLEEELRRRLTE

SEQ ID NO: 29 - protein, 15 aa, Artificial Sequence
  synthetic peptide
MSRLEEELRRRLTEP

SEQ ID NO: 30 - protein, 16 aa, Artificial Sequence
  synthetic peptide
MSSRLEEELRRRLTEP

SEQ ID NO: 31 - protein, 13 aa, Artificial Sequence
  synthetic peptide
  MISC_FEATURE (1)..(1): Xaa is G or S or P
  MISC_FEATURE (2)..(2): Xaa is R or G
  MISC_FEATURE (5)..(5): Xaa is E or Q
  MISC_FEATURE (7)..(7): Xaa is L or I
  MISC_FEATURE (12)..(12): Xaa is S or T or P or A
  MISC_FEATURE (13)..(13): Xaa is P or A or S or no amino acid
XXLEXEXRRRLXX

SEQ ID NO: 32 - protein, 12 aa, Artificial Sequence
  synthetic peptide
GRLEEELRRRLS

SEQ ID NO: 33 - protein, 15 aa, Artificial Sequence
  synthetic peptide
MSGRLEEELRRRLSP

SEQ ID NO: 34 - protein, 16 aa, Artificial Sequence
  synthetic peptide
SDSGLEQELRRRLSPG

SEQ ID NO: 35 - protein, 16 aa, Artificial Sequence
  synthetic peptide
PDGGLEQELRRRLTAP

SEQ ID NO: 36 - protein, 16 aa, Artificial Sequence
  synthetic peptide
PSGGLEQELRRRLTAP

SEQ ID NO: 37 - protein, 16 aa, Artificial Sequence
  synthetic peptide
DSPGLEQELRRRLTAP

SEQ ID NO: 38 - protein, 16 aa, Artificial Sequence
  synthetic peptide
PDSGLEQELRRRLTPA

SEQ ID NO: 39 - protein, 17 aa, Artificial Sequence
  synthetic peptide
SPSGLEEELRRRLTAEP

SEQ ID NO: 40 - protein, 14 aa, Artificial Sequence
  synthetic peptide
GPSGLEQELRRRLT

SEQ ID NO: 41 - protein, 17 aa, Artificial Sequence
  synthetic peptide
GPSGLEQELRRRLTAAS

SEQ ID NO: 42 - protein, 16 aa, Artificial Sequence
  synthetic peptide
SPSRLEEELRRRLPSK

SEQ ID NO: 43 - protein, 16 aa, Artificial Sequence
  synthetic peptide
SPSGLEQELRRRLTPS

SEQ ID NO: 44 - protein, 16 aa, Artificial Sequence
  synthetic peptide
SPGRLEQEIRRRLSPS

SEQ ID NO: 45 - protein, 16 aa, Artificial Sequence
  synthetic peptide
PSGRLEEELRRRLSPS

SEQ ID NO: 46 - protein, 14 aa, Artificial Sequence
  synthetic peptide
PSGRLEEELRRRLS

SEQ ID NO: 47 - protein, 14 aa, Artificial Sequence
  synthetic peptide
PSGRLEEELRRRLA

SEQ ID NO: 48 - protein, 15 aa, Artificial Sequence
  synthetic peptide
PSGRLEEELRRRLSP

SEQ ID NO: 49 - protein, 13 aa, Artificial Sequence
  synthetic peptide
  MISC_FEATURE (1)..(1): Xaa is S or G or P
  MISC_FEATURE (2)..(2): Xaa is R or G or P
  MISC_FEATURE (5)..(5): Xaa is E or Q
  MISC_FEATURE (12)..(12): Xaa is S or T or D or E
  MISC_FEATURE (13)..(13): Xaa is P or A or D or no amino acid
XXLEXELRRRLXX

SEQ ID NO: 50 - protein, 16 aa, Artificial Sequence
  synthetic peptide
PDSGLEQELRRRLSPG

SEQ ID NO: 51 - protein, 16 aa, Artificial Sequence
  synthetic peptide
PDSGLEQELRRRLTAP

SEQ ID NO: 52 - protein, 16 aa, Artificial Sequence
  synthetic peptide
PSSGLEQELRRRLTAP

SEQ ID NO: 53 - protein, 16 aa, Artificial Sequence
  synthetic peptide
DPSGLEQELRRRLTAP

SEQ ID NO: 54 - protein, 16 aa, Artificial Sequence
  synthetic peptide
DSGPLEQELRRRLTAP

SEQ ID NO: 55 - protein, 17 aa, Artificial Sequence
  synthetic peptide
SPSRLEEELRRRLTAEP

SEQ ID NO: 56 - protein, 16 aa, Artificial Sequence
  synthetic peptide
SPSGLEEELRRRLTAP

SEQ ID NO: 57 - protein, 16 aa, Artificial Sequence
  synthetic peptide
SPSGLEEELRRRLDAP

SEQ ID NO: 58 - protein, 16 aa, Artificial Sequence
  synthetic peptide
SPSGLEEELRRRLEAP

SEQ ID NO: 59 - protein, 16 aa, Artificial Sequence
  synthetic peptide
SPSGLEEELRRRLTDP

SEQ ID NO: 60 - protein, 17 aa, Artificial Sequence
  synthetic peptide
SPSGLEEELRRRLTADP

SEQ ID NO: 61 - protein, 13 aa, Artificial Sequence
  synthetic peptide
  MISC_FEATURE (1)..(1): Xaa is G or S
  MISC_FEATURE (2)..(2): Xaa is R or G or A or E
  MISC_FEATURE (3)..(3): Xaa is L or V
  MISC_FEATURE (4)..(4): Xaa is E or Q
  MISC_FEATURE (5)..(5): Xaa is E or Q
  MISC_FEATURE (6)..(6): Xaa is E or Q
  MISC_FEATURE (7)..(7): Xaa is L or I or V
  MISC_FEATURE (8)..(8): Xaa is R or A or Q or E
  MISC_FEATURE (9)..(9): Xaa is R or A or Q or E
  MISC_FEATURE (12)..(12): Xaa is S or T or L or no amino acid
  MISC_FEATURE (13)..(13): Xaa is K or P or S or no amino acid
XXXXXXXXXRLXX

SEQ ID NO: 62 - protein, 16 aa, Artificial Sequence
  synthetic peptide
DSGRLEEELRRRLSKG

SEQ ID NO: 63 - protein, 16 aa, Artificial Sequence
  synthetic peptide
DSGRLEEELRRRLSPG

SEQ ID NO: 64 - protein, 16 aa, Artificial Sequence
  synthetic peptide
SDSGLEEELRRRLSPG

SEQ ID NO: 65 - protein, 16 aa, Artificial Sequence
  synthetic peptide
SDSGVEEELRRRLSPG

SEQ ID NO: 66 - protein, 16 aa, Artificial Sequence
  synthetic peptide
SDSAVEEELRRRLSPG

SEQ ID NO: 67 - protein, 16 aa, Artificial Sequence
  synthetic peptide
SDSGLQEELRRRLSPG

SEQ ID NO: 68 - protein, 16 aa, Artificial Sequence
  synthetic peptide
SDSGLEEQLRRRLSPG

SEQ ID NO: 69 - protein, 16 aa, Artificial Sequence
  synthetic peptide
SDSGLEEEIRRRLSPG

SEQ ID NO: 70 - protein, 16 aa, Artificial Sequence
  synthetic peptide
SDSGLEEEVRRRLSPG

SEQ ID NO: 71 - protein, 16 aa, Artificial Sequence
  synthetic peptide
DSGELEEELRRRLSPG

SEQ ID NO: 72 - protein, 16 aa, Artificial Sequence
  synthetic peptide
DSGRLEQELRRRLSPG

SEQ ID NO: 73 - protein, 18 aa, Artificial Sequence
  synthetic peptide
QQDSGRLEEEIRRRLSPG

SEQ ID NO: 74 - protein, 16 aa, Artificial Sequence
  synthetic peptide
DSGRLEQEIRRRLSPG

SEQ ID NO: 75 - protein, 16 aa, Artificial Sequence
  synthetic peptide
DSGRLEQEIARRLSPG

SEQ ID NO: 76 - protein, 16 aa, Artificial Sequence
  synthetic peptide
DSGRLEQEIQRRLSPG

SEQ ID NO: 77 - protein, 16 aa, Artificial Sequence
  synthetic peptide
DSGRLEQEIERRLSPG

SEQ ID NO: 78 - protein, 16 aa, Artificial Sequence
  synthetic peptide
DSGRLEQEIRARLSPG

SEQ ID NO: 79 - protein, 16 aa, Artificial Sequence
  synthetic peptide
DSGRLEQEIRQRLSPG

SEQ ID NO: 80 - protein, 16 aa, Artificial Sequence
  synthetic peptide
DSGRLEQEIRERLSPG

SEQ ID NO: 81 - protein, 13 aa, Artificial Sequence
  synthetic peptide
GPSRLEEELRRRL

SEQ ID NO: 82 - protein, 15 aa, Artificial Sequence
  synthetic peptide
MSGLEQELRRRLTPS

SEQ ID NO: 83 - protein, 16 aa, Artificial Sequence
  synthetic peptide
MSGRLEEELRRRLSPS

SEQ ID NO: 84 - protein, 16 aa, Artificial Sequence
  synthetic peptide
SPSAVEEELRRRLSPS

SEQ ID NO: 85 - protein, 14 aa, Artificial Sequence
  synthetic peptide
GPSAVEEELRRRLS

SEQ ID NO: 86 - protein, 16 aa, Artificial Sequence
  synthetic peptide
MPSGLEQELRRRLTPS

SEQ ID NO: 87 - protein, 16 aa, Artificial Sequence
  synthetic peptide
MSSGLEQELRRRLTPS

SEQ ID NO: 88 - protein, 17 aa, Artificial Sequence
  synthetic peptide
MPSGRLEEELRRRLSPS

SEQ ID NO: 89 - protein, 15 aa, Artificial Sequence
  synthetic peptide
MSGRLEEELRRRLSP

SEQ ID NO: 90 - protein, 16 aa, Artificial Sequence
  synthetic peptide
DSMRLEEELRRRLSKG

SEQ ID NO: 91 - protein, 16 aa, Artificial Sequence
  synthetic peptide
DSMRLEEELRRRLSPG

SEQ ID NO: 92 - protein, 15 aa, Artificial Sequence
  synthetic peptide
SDSGEEELRRRLSPG

SEQ ID NO: 93 - protein, 14 aa, Artificial Sequence
  synthetic peptide
SDSGEELRRRLSPG

SEQ ID NO: 94 - protein, 15 aa, Artificial Sequence
  synthetic peptide
DSGRLEEELRRRSPG

SEQ ID NO: 95 - protein, 14 aa, Artificial Sequence
  synthetic peptide
DSGRLEEELRRSPG

SEQ ID NO: 96 - protein, 13 aa, Artificial Sequence
  synthetic peptide
DSGRLEEELRSPG

SEQ ID NO: 97 - protein, 16 aa, Artificial Sequence
  synthetic peptide
SDSGLEEEARRRLSPG

SEQ ID NO: 98 - protein, 16 aa, Artificial Sequence
  synthetic peptide
SDSGAEEELRRRLSPG

SEQ ID NO: 99 - protein, 16 aa, Artificial Sequence
  synthetic peptide
DSGALEEELRRRLSPG

SEQ ID NO: 100 - protein, 16 aa, Artificial Sequence
  synthetic peptide
DSGALEQEIRRRLSPG

SEQ ID NO: 101 - protein, 16 aa, Artificial Sequence
  synthetic peptide
DSGRLEQEIRRALSPG

SEQ ID NO: 102 - protein, 16 aa, Artificial Sequence
  synthetic peptide
DSGRLEQEIRRQLSPG

SEQ ID NO: 103 - protein, 16 aa, Artificial Sequence
  synthetic peptide
DSGRLEQEIRRELSPG

SEQ ID NO: 104 - protein, 16 aa, Artificial Sequence
  synthetic peptide
PDSGLEQELRRRLPTA

SEQ ID NO: 105 - protein, 16 aa, Artificial Sequence
  synthetic peptide
DPSGLEQELRRRLPTA

SEQ ID NO: 106 - protein, 16 aa, Artificial Sequence
  synthetic peptide
DSPGLEQELRRRLPTA

SEQ ID NO: 107 - protein, 16 aa, Artificial Sequence
  synthetic peptide
DSGPLEQELRRRLPTA

SEQ ID NO: 108 - protein, 13 aa, Artificial Sequence
  synthetic peptide
GPSGLEQELRRRL

SEQ ID NO: 109 - protein, 15 aa, Artificial Sequence
  synthetic peptide
MSAVEEELRRRLSPS

SEQ ID NO: 110 - protein, 15 aa, Artificial Sequence
  synthetic peptide
MSGLEQELRRRLTPS

SEQ ID NO: 111 - protein, 15 aa, Artificial Sequence
  synthetic peptide
MSAVEEELRRRLSPS

SEQ ID NO: 112 - protein, 16 aa, Artificial Sequence
  synthetic peptide
MPSAVEEELRRRLSPS

SEQ ID NO: 113 - protein, 16 aa, Artificial Sequence
  synthetic peptide
MSSAVEEELRRRLSPS

SEQ ID NO: 114 - protein, 14 aa, Artificial Sequence
  synthetic peptide
PSGRLEEELRRRLP

SEQ ID NO: 115 - protein, 13 aa, Artificial Sequence
  antibody CDR
GVTISALNAMAMG

SEQ ID NO: 116 - protein, 9 aa, Artificial Sequence
  antibody CDR
AVSERGNAM

SEQ ID NO: 117 - protein, 11 aa, Artificial Sequence
  antibody CDR
LEDRVDSFHDY

SEQ ID NO: 118 - protein, 13 aa, Artificial Sequence
  antibody CDR
GVTISALNAMAMG

SEQ ID NO: 119 - protein, 9 aa, Artificial Sequence
  antibody CDR
AVSSRGNAM

SEQ ID NO: 120 - protein, 11 aa, Artificial Sequence
  antibody CDR
LEDRVDSFHDY

SEQ ID NO: 121 - protein, 13 aa, Artificial Sequence
  antibody CDR
GVTVSALNAMAMG

SEQ ID NO: 122 - protein, 9 aa, Artificial Sequence
  antibody CDR
AVSERGNAM

SEQ ID NO: 123 - protein, 11 aa, Artificial Sequence
  antibody CDR
LEDRVDSFHDY

SEQ ID NO: 124 - protein, 25 aa, Artificial Sequence
  antibody FR
  MISC_FEATURE (5)..(5): Xaa is Q, V, E, or L
  MISC_FEATURE (13)..(13): Xaa is Q or P
  MISC_FEATURE (18)..(18): Xaa is L or M
EVQLXESGGGLVXPGGSXRLSCTAS

SEQ ID NO: 125 - protein, 25 aa, Artificial Sequence
  antibody FR
EVQLQESGGGLVQPGGSLRLSCTAS

SEQ ID NO: 126 - protein, 14 aa, Artificial Sequence
  antibody FR
  MISC_FEATURE (5)..(5): Xaa is A or R
  MISC_FEATURE (9)..(9): Xaa is R or E
WYRQXPGEXRVMVA

SEQ ID NO: 127 - protein, 14 aa, Artificial Sequence
  antibody FR
WYRQAPGERRVMVA

SEQ ID NO: 128 - protein, 14 aa, Artificial Sequence
  antibody FR
WYRQAPGEERVMVA

SEQ ID NO: 129 - protein, 39 aa, Artificial Sequence
  antibody FR
  MISC_FEATURE (28)..(28): Xaa is K or Q
  MISC_FEATURE (32)..(32): Xaa is T or M
YRESVQGRFTVTRDFTNKMVSLQMDNLXPEDXAVYYCHV

SEQ ID NO: 130 - protein, 39 aa, Artificial Sequence
  antibody FR
YRESVQGRFTVTRDFTNKMVSLQMDNLKPEDTAVYYCHV

SEQ ID NO: 131 - protein, 11 aa, Artificial Sequence
  antibody FR
  MISC_FEATURE (5)..(5): Xaa is T or I
WGQGXQVTVSS

SEQ ID NO: 132 - protein, 11 aa, Artificial Sequence
  antibody FR
WGQGTQVTVSS

SEQ ID NO: 133 - protein, 122 aa, Artificial Sequence
  Camelid VHH domain
EVQLQESGGGLVQPGGSLRLSCTASGVTISALNAMAMGWYRQAPGERRVMVAAVSERGNAMYRESVQGRFTVTRDFTNKMVSLQMDNLKPEDTAVYYCHVLEDRVDSFHDYWGQGTQVTVSS

SEQ ID NO: 134 - protein, 122 aa, Artificial Sequence
  Camelid VHH domain
EVQLQESGGGLVQPGGSLRLSCTASGVTISALNAMAMGWYRQAPGEERVMVAAVSSRGNAMYRESVQGRFTVTRDFTNKMVSLQMDNLKPEDTAVYYCHVLEDRVDSFHDYWGQGTQVTVSS

SEQ ID NO: 135 - protein, 122 aa, Artificial Sequence
  Camelid VHH domain
EVQLQESGGGLVQPGGSLRLSCTASGVTISALNAMAMGWYRQAPGEERVMVAAVSERGNAMYRESVQGRFTVTRDFTNKMVSLQMDNLKPEDTAVYYCHVLEDRVDSFHDYWGQGTQVTVSS

SEQ ID NO: 136 - protein, 122 aa, Artificial Sequence
  Camelid VHH domain
EVQLQESGGGLVQPGGSLRLSCTASGVTISALNAMAMGWYRQAPGERRVMVAAVSSRGNAMYRESVQGRFTVTRDFTNKMVSLQMDNLKPEDTAVYYCHVLEDRVDSFHDYWGQGTQVTVSS

SEQ ID NO: 137 - protein, 122 aa, Artificial Sequence
  Camelid VHH domain
EVQLVESGGGLVPPGGSMRLSCTASGVTVSALNAMAMGWYRQRPGERRVMVAAVSERGNAMYRESVQGRFTVTRDFTNKMVSLQMDNLQPEDMAVYYCHVLEDRVDSFHDYWGQGIQVTVSS

SEQ ID NO: 138 - protein, 122 aa, Artificial Sequence
  Camelid VHH domain
EVQLVESGGGLVPPGGSMRLSCTAPGVTVSALNAMAMGWYRQRPGERRVMVAAVSERGNAMYRESVQGRFTVTRDFTNKMVSLQMDNLQPEDMAVYYCHVLEDRVDSFHDYWGQGIQVTVSS

SEQ ID NO: 139 - protein, 122 aa, Artificial Sequence
  Camelid VHH domain
EVQLVESGGGVVQPGGSLRLSCTASGVTISALNAMAMGWYRQAPGERRVMVAAVSERGNAMYRESVQGRFTVTRDFTNKMVSLQMDNLKPEDTAVYYCHVLEDRVDSFHDYWGQGTQVTVSS

SEQ ID NO: 140 - protein, 122 aa, Artificial Sequence
  Camelid VHH domain
EVQLVESGGGLVQPGGSLRLSCTASGVTISALNAMAMGWYRQAPGERRVMVAAVSERGNAMYRESVQGRFTVTRDFTNKMVSLQMDNLKPEDTAVYYCHVLEDRVDSFHDYWGQGTQVTVSS

SEQ ID NO: 141 - protein, 122 aa, Artificial Sequence
  Camelid VHH domain
EVQLEESGGGLVQPGGSLRLSCTASGVTISALNAMAMGWYRQAPGERRVMVAAVSERGNAMYRESVQGRFTVTRDFTNKMVSLQMDNLKPEDTAVYYCHVLEDRVDSFHDYWGQGTQVTVSS

SEQ ID NO: 142 - protein, 122 aa, Artificial Sequence
  Camelid VHH domain
EVQLLESGGGLVQPGGSLRLSCTASGVTISALNAMAMGWYRQAPGERRVMVAAVSERGNAMYRESVQGRFTVTRDFTNKMVSLQMDNLKPEDTAVYYCHVLEDRVDSFHDYWGQGTQVTVSS

SEQ ID NO: 143 - protein, 10 aa, Artificial Sequence
  antibody CDR
GTMSAINALN

SEQ ID NO: 144 - protein, 9 aa, Artificial Sequence
  antibody CDR
AITDNGNAH

SEQ ID NO: 145 - protein, 12 aa, Artificial Sequence
  antibody CDR
LEEEKLGVWVDY

SEQ ID NO: 146 - protein, 10 aa, Artificial Sequence
  antibody CDR
GTMSAINALN

SEQ ID NO: 147 - protein, 9 aa, Artificial Sequence
  antibody CDR
AITDNGNAH

SEQ ID NO: 148 - protein, 11 aa, Artificial Sequence
  antibody CDR
LEEKLGAWVDY

SEQ ID NO: 149 - protein, 10 aa, Artificial Sequence
  antibody CDR
GTMSAINALN

SEQ ID NO: 150 - protein, 9 aa, Artificial Sequence
  antibody CDR
AITDNGNAH

SEQ ID NO: 151 - protein, 12 aa, Artificial Sequence
  antibody CDR
LEKEKLGVWVDY

SEQ ID NO: 152 - protein, 25 aa, Artificial Sequence
  antibody FR
  MISC_FEATURE (5)..(5): Xaa is V or L
EVQLXESGGGLVQPGGSLTLSCAAS

SEQ ID NO: 153 - protein, 14 aa, Artificial Sequence
  antibody FR
  MISC_FEATURE (5)..(5): Xaa is P or A
WYRQXPGKERKMVA

SEQ ID NO: 154 - protein, 39 aa, Artificial Sequence
  antibody FR
  MISC_FEATURE (28)..(28): Xaa is K or E
YADSVKGRFTISRDNARNMVFLQMNSLXPDDTAVYYCHY

SEQ ID NO: 155 - protein, 11 aa, Artificial Sequence
  antibody FR
WGQGTQVTVSS

SEQ ID NO: 156 - protein, 120 aa, Artificial Sequence
  Camelid VHH domain
EVQLVESGGGLVQPGGSLTLSCAASGTMSAINALNWYRQPPGKERKMVAAITDNGNAHYADSVKGRFTISRDNARNMVFLQMNSLKPDDTAVYYCHYLEEEKLGVWVDYWGQGTQVTVSS

SEQ ID NO: 157 - protein, 119 aa, Artificial Sequence
  Camelid VHH domain
EVQLLESGGGLVQPGGSLTLSCAASGTMSAINALNWYRQAPGKERKMVAAITDNGNAHYADSVKGRFTISRDNARNMVFLQMNSLEPDDTAVYYCHYLEEKLGAWVDYWGQGTQVTVSS

SEQ ID NO: 158 - protein, 120 aa, Artificial Sequence
  Camelid VHH domain
EVQLVESGGGLVQPGGSLTLSCAASGTMSAINALNWYRQPPGKERKMVAAITDNGNAHYADSVKGRFTISRDNARNMVFLQMNSLKPDDTAVYYCHYLEKEKLGVWVDYWGQGTQVTVSS

SEQ ID NO: 159 - protein, 15 aa, Artificial Sequence
  linker
GGGGSGGGGSGGGGS

SEQ ID NO: 160 - protein, 8 aa, Artificial Sequence
  FLAG-tag
DYKDDDDK

SEQ ID NO: 161 - protein, 10 aa, Artificial Sequence
  Myc-tag
EQKLISEEDL

SEQ ID NO: 162 - protein, 9 aa, Artificial Sequence
  HA-tag
YPYDVPDYA

SEQ ID NO: 163 - protein, 11 aa, Artificial Sequence
  VSV-G-tag
YTDIEMNRLGK

SEQ ID NO: 164 - protein, 11 aa, Artificial Sequence
  HSV-tag
QPELAPEDPED

SEQ ID NO: 165 - protein, 14 aa, Artificial Sequence
  V5-tag
GKPIPNPLLGLDST

SEQ ID NO: 166 - protein, 12 aa, Artificial Sequence
  SPOT-tag
PDRVRAVSHWSS

SEQ ID NO: 167 - protein, 12 aa, Artificial Sequence
  BC2 tag
PDRKAAVSHWQQ

SEQ ID NO: 168 - protein, 4 aa, Artificial Sequence
  EPEA tag
EPEA

SEQ ID NO: 169 - protein, 15 aa, Artificial Sequence
  synthetic peptide
GPSGLEQELRRRLTA

SEQ ID NO: 170 - protein, 16 aa, Artificial Sequence
  synthetic peptide
SPSGLEQELRRRLTDP

SEQ ID NO: 171 - protein, 17 aa, Artificial Sequence
  synthetic peptide
SPSGLEQELRRRLTADP

SEQ ID NO: 172 - protein, 17 aa, Artificial Sequence
  synthetic peptide
SPSGLEQELRRRLTAEP

SEQ ID NO: 173 - protein, 16 aa, Artificial Sequence
  synthetic peptide
DSPGLEQELRRRLTAP

SEQ ID NO: 174 - protein, 16 aa, Artificial Sequence
  synthetic peptide
SPSGLEQELRRRLSPS

SEQ ID NO: 175 - protein, 122 aa, Artificial Sequence
  Camelid VHH domain
EVQLQESGGGLVQPGGSLRLSCTASGVTISALNAMAMGWYRQAPGERRVMVAAVSDRGNAMYRESVQGRFTVTRDFTNKMVSLQMDNLKPEDTAVYYCHVLEDRVDSFHDYWGQGTQVTVSS

SEQ ID NO: 176 - protein, 122 aa, Artificial Sequence
  Camelid VHH domain
EVQLQESGGGLVQPGGSLRLSCTASGVTISALNAMAMGWYRQAPGERRVMVAAVSNRGNAMYRESVQGRFTVTRDFTNKMVSLQMDNLKPEDTAVYYCHVLEDRVDSFHDYWGQGTQVTVSS

SEQ ID NO: 177 - protein, 122 aa, Artificial Sequence
  Camelid VHH domain
EVQLQESGGGLVQPGGSLRLSCTASGVTISALNAMAMGWYRQAPGERRVMVAAVSHRGNAMYRESVQGRFTVTRDFTNKMVSLQMDNLKPEDTAVYYCHVLEDRVDSFHDYWGQGTQVTVSS

SEQ ID NO: 178 - protein, 8 aa, Artificial Sequence
  Strep-tag
WSHPQFEK

SEQ ID NO: 179 - protein, 15 aa, Artificial Sequence
  synthetic peptide
  MOD_RES (1)..(1): ACETYLATION
  MOD_RES (15)..(15): AMIDATION
PSRLEEELRRRLTEP

SEQ ID NO: 180 - protein, 490 aa, Artificial Sequence
  fusion protein
MPSRLEEELRRRLTEPDYKDDDDKGSTRSVSSSSYRRMFGGSGTSSRPSSNRSYVTTSTRTYSLGSALRPSTSRSLYSSSPGGAYVTRSSAVRLRSSVPGVRLLQDSVDFSLADAINTEFKNTRTNEKVELQELNDRFANYIDKVRFLEQQNKILLAELEQLKGQGKSRLGDLYEEEMRELRRQVDQLTNDKARVEVERDNLAEDIMRLREKLQEEMLQREEAESTLQSFRQDVDNASLARLDLERKVESLQEEIAFLKKLHDEEIQELQAQIQEQHVQIDVDVSKPDLTAALRDVRQQYESVAAKNLQEAEEWYKSKFADLSEAANRNNDALRQAKQESNEYRRQVQSLTCEVDALKGTNESLERQMREMEENFALEAANYQDTIGRLQDEIQNMKEEMARHLREYQDLLNVKMALDIEIATYRKLLEGEESRISLPLPTFSSLNLRETNLESLPLVDTHSKRTLLIKTVETRDGQVINETSQHHDDLE

SEQ ID NO: 181 - protein, 489 aa, Artificial Sequence
  fusion protein
MSGRLEEELRRRLSPDYKDDDDKGSTRSVSSSSYRRMFGGSGTSSRPSSNRSYVTTSTRTYSLGSALRPSTSRSLYSSSPGGAYVTRSSAVRLRSSVPGVRLLQDSVDFSLADAINTEFKNTRTNEKVELQELNDRFANYIDKVRFLEQQNKILLAELEQLKGQGKSRLGDLYEEEMRELRRQVDQLTNDKARVEVERDNLAEDIMRLREKLQEEMLQREEAESTLQSFRQDVDNASLARLDLERKVESLQEEIAFLKKLHDEEIQELQAQIQEQHVQIDVDVSKPDLTAALRDVRQQYESVAAKNLQEAEEWYKSKFADLSEAANRNNDALRQAKQESNEYRRQVQSLTCEVDALKGTNESLERQMREMEENFALEAANYQDTIGRLQDEIQNMKEEMARHLREYQDLLNVKMALDIEIATYRKLLEGEESRISLPLPTFSSLNLRETNLESLPLVDTHSKRTLLIKTVETRDGQVINETSQHHDDLE

SEQ ID NO: 182 - protein, 291 aa, Artificial Sequence
  fusion protein
MKSFITRNKTAILATVAATGTAIGAYYYYGNSPVATMVSKGEELFTGVVPILVELDGDVNGHKFSVSGEGEGDATYGKLTLKFICTTGKLPVPWPTLVTTLTYGVQCFSRYPDHMKQHDFFKSAMPEGYVQERTIFFKDDGNYKTRAEVKFEGDTLVNRIELKGIDFKEDGNILGHKLEYNYNSHNVYIMADKQKNGIKVNFKIRHNIEDGSVQLADHYQQNTPIGDGPVLLPDNHYLSTQSKLSKDPNEKRDHMVLLEFVTAAGITLGMDELYKGSPSRLEEELRRRLTE

SEQ ID NO: 183 - protein, 291 aa, Artificial Sequence; identical to SEQ ID NO: 182
  fusion protein

SEQ ID NO: 184 - protein, 350 aa, Artificial Sequence
  fusion protein
METDTLLLWVLLLWVPGSTGDYPYDVPDYASNGTSKGEELFTGVVPILVELDGDVNGHKFSVSGEGEGDATYGKLTLKFICTTGKLPVPWPTLVTTLTYGVQCFSRYPDHMKQHDFFKSAMPEGYVQERTIFFKDDGNYKTRAEVKFEGDTLVNRIELKGIDFKEDGNILGHKLEYNYNSHNVYIMADKQKNGIKVNFKIRHNIEDGSVQLADHYQQNTPIGDGPVLLPDNHYLSTQSALSKDPNEKRDHMVLKEFVTAAGITLGMDELYKGSPSRLEEELRRRLTEPGDEQKLISEEDLNAVGQDTQEVIVVPHSLPFKVVVISAILALVVLTIISLIILIMLWQKKPR

SEQ ID NO: 185 - protein, 382 aa, Artificial Sequence
  fusion protein
MGSGDASDSEVQLQESGGGLVQPGGSLRLSCTASGVTISALNAMAMGWYRQAPGERRVMVAAVSERGNAMYRESVQGRFTVTRDFTNKMVSLQMDNLKPEDTAVYYCHVLEDRVDSFHDYWGQGTQVTVSSEPKTPKPQTSGSTGENVATMVSKGEAVIKEFMRFKVHMEGSMNGHEFEIEGEGEGRPYEGTQTAKLKVTKGGPLPFSWDILSPQFMYGSRAFIKHPADIPDYYKQSFPEGFKWERVMNFEDGGAVTVTQDTSLEDGTLIYKVKLRGTNFPPDGPVMQKKTMGWEASTERLYPEDGVLKGDIKMALRLKDGGRYLADFKTTYKAKKPVQMPGAYNVDRKLDITSHNEDYTVVEQYERSEGRHSTGGMDELYK

SEQ ID NO: 186 - protein, 239 aa, Artificial Sequence
  EGFP
MVSKGEELFTGVVPILVELDGDVNGHKFSVSGEGEGDATYGKLTLKFICTTGKLPVPWPTLVTTLTYGVQCFSRYPDHMKQHDFFKSAMPEGYVQERTIFFKDDGNYKTRAEVKFEGDTLVNRIELKGIDFKEDGNILGHKLEYNYNSHNVYIMADKQKNGIKVNFKIRHNIEDGSVQLADHYQQNTPIGDGPVLLPDNHYLSTQSALSKDPNEKRDHMVLLEFVTAAGITLGMDELYK

SEQ ID NO: 187 - protein, 255 aa, Artificial Sequence
  fusion protein
MVSKGEELFTGVVPILVELDGDVNGHKFSVSGEGEGDATYGKLTLKFICTTGKLPVPWPTLVTTLTYGVQCFSRYPDHMKQHDFFKSAMPEGYVQERTIFFKDDGNYKTRAEVKFEGDTLVNRIELKGIDFKEDGNILGHKLEYNYNSHNVYIMADKQKNGIKVNFKIRHNIEDGSVQLADHYQQNTPIGDGPVLLPDNHYLSTQSALSKDPNEKRDHMVLLEFVTAAGITLGMDELYKGSPSRLEEELRRRLTE

SEQ ID NO: 188 - protein, 255 aa, Artificial Sequence
  fusion protein
MPSRLEEELRRRLTEPMVSKGEELFTGVVPILVELDGDVNGHKFSVSGEGEGDATYGKLTLKFICTTGKLPVPWPTLVTTLTYGVQCFSRYPDHMKQHDFFKSAMPEGYVQERTIFFKDDGNYKTRAEVKFEGDTLVNRIELKGIDFKEDGNILGHKLEYNYNSHNVYIMADKQKNGIKVNFKIRHNIEDGSVQLADHYQQNTPIGDGPVLLPDNHYLSTQSALSKDPNEKRDHMVLLEFVTAAGITLGMDELYK

SEQ ID NO: 189 - protein, 558 aa, Artificial Sequence
  fusion protein
MSKHHHHSNHHRHNHHHHSGNHHHSGSAAGGEEDKKPAGGEGGGAHINLKVKGQDGNEVFFRIKRSTQLKKLMNAYCDRQSVDMTAIAFLFDGRRLRAEQTPDELEMEDGDEIDAMLHQTGGASDYKDDDDKGSTGDYPYDVPDYASNGTKTEEGKLVIWINGDKGYNGLAEVGKKFEKDTGIKVTVEHPDKLEEKFPQVAATGDGPDIIFWAHDRFGGYAQSGLLAEITPDKAFQDKLYPFTWDAVRYNGKLIAYPIAVEALSLIYNKDLLPNPPKTWEEIPALDKELKAKGKSALMFNLQEPYFTWPLIAADGGYAFKYENGKYDIKDVGVDNAGAKAGLTFLVDLIKNKHMNADTDYSIAEAAFNKGETAMTINGPWAWSNIDTSKVNYGVTVLPTFKGQPSKPFVGVLSAGINAASPNKELAKEFLENYLLTDEGLEAVNKDKPLGAVALKSYEEELAKDPRIAATMENAQKGEIMPNIPQMSAFWYAVRTAVINAASGRQTVDEALKDAQTNGSVSAGDEQKLISEEDLNAVGQDTASTPSRLEEELRRRLTE

SEQ ID NO: 190 - protein, 259 aa, Artificial Sequence
  fusion protein
MPSRLEEELRRRLTEPSKGEELFTGTVPIKVELDGDVNGHKFSVRGEGEGDATEGKLTLKFICTTGKLPVPWPTLVTTLTYGVQCFSRYPDHMKRHDFFKSAMPEGYVQERTIEFKDDGTYKTRAEVKFEGDTLVNRIELKGNDFKEDGNILGHKLEYNHNSHNVRIEADKQKNGIKANFKIRHNVEDGSQQEADHKQQNTPIGDGPVRLPDNHYLSTQTTLSKDPNEKRDHMVLKEFVTAAGITKGEDERDKHHHHHH

SEQ ID NO: 191 - protein, 258 aa, Artificial Sequence
  fusion protein
MSGRLEEELRRRLSPSKGEELFTGTVPIKVELDGDVNGHKFSVRGEGEGDATEGKLTLKFICTTGKLPVPWPTLVTTLTYGVQCFSRYPDHMKRHDFFKSAMPEGYVQERTIEFKDDGTYKTRAEVKFEGDTLVNRIELKGNDFKEDGNILGHKLEYNHNSHNVRIEADKQKNGIKANFKIRHNVEDGSQQEADHKQQNTPIGDGPVRLPDNHYLSTQTTLSKDPNEKRDHMVLKEFVTAAGITKGEDERDKHHHHHH

SEQ ID NO: 192 - protein, 381 aa, Artificial Sequence
  fusion protein
MSKHHHHSNHHRHNHHHHSGNHHHSGSAAGGEEDKKPAGGEGGGAHINLKVKGQDGNEVFFRIKRSTQLKKLMNAYCDRQSVDMTAIAFLFDGRRLRAEQTPDELEMEDGDEIDAMLHQTGGGSKGEELFTGTVPIKVELDGDVNGHKFSVRGEGEGDATEGKLTLKFICTTGKLPVPWPTLVTTLTYGVQCFSRYPDHMKRHDFFKSAMPEGYVQERTIEFKDDGTYKTRAEVKFEGDTLVNRIELKGNDFKEDGNILGHKLEYNHNSHNVRIEADKQKNGIKANFKIRHNVEDGSQQEADHKQQNTPIGDGPVRLPDNHYLSTQTTLSKDPNEKRDHMVLKEFVTAAGITKGEDERDKGSGNSDGPSRLEEELRRRLTE

SEQ ID NO: 193 - protein, 382 aa, Artificial Sequence
  fusion protein
MSKHHHHSNHHRHNHHHHSGNHHHSGSAAGGEEDKKPAGGEGGGAHINLKVKGQDGNEVFFRIKRSTQLKKLMNAYCDRQSVDMTAIAFLFDGRRLRAEQTPDELEMEDGDEIDAMLHQTGGGSKGEELFTGTVPIKVELDGDVNGHKFSVRGEGEGDATEGKLTLKFICTTGKLPVPWPTLVTTLTYGVQCFSRYPDHMKRHDFFKSAMPEGYVQERTIEFKDDGTYKTRAEVKFEGDTLVNRIELKGNDFKEDGNILGHKLEYNHNSHNVRIEADKQKNGIKANFKIRHNVEDGSQQEADHKQQNTPIGDGPVRLPDNHYLSTQTTLSKDPNEKRDHMVLKEFVTAAGITKGEDERDKGSGNSDGMSGRLEEELRRRLSP

SEQ ID NO: 194 - protein, 382 aa, Artificial Sequence
  fusion protein
MSKHHHHSNHHRHNHHHHSGNHHHSGSAAGGEEDKKPAGGEGGGAHINLKVKGQDGNEVFFRIKRSTQLKKLMNAYCDRQSVDMTAIAFLFDGRRLRAEQTPDELEMEDGDEIDAMLHQTGGSGDASDSPSRLEEELRRRLTEPSKGEELFTGTVPIKVELDGDVNGHKFSVRGEGEGDATEGKLTLKFICTTGKLPVPWPTLVTTLTYGVQCFSRYPDHMKRHDFFKSAMPEGYVQERTIEFKDDGTYKTRAEVKFEGDTLVNRIELKGNDFKEDGNILGHKLEYNHNSHNVRIEADKQKNGIKANFKIRHNVEDGSQQEADHKQQNTPIGDGPVRLPDNHYLSTQTTLSKDPNEKRDHMVLKEFVTAAGITKGEDERDKA

SEQ ID NO: 195 - protein, 382 aa, Artificial Sequence
  fusion protein
MSKHHHHSNHHRHNHHHHSGNHHHSGSAAGGEEDKKPAGGEGGGAHINLKVKGQDGNEVFFRIKRSTQLKKLMNAYCDRQSVDMTAIAFLFDGRRLRAEQTPDELEMEDGDEIDAMLHQTGGSGDASDSMSGRLEEELRRRLSPSKGEELFTGTVPIKVELDGDVNGHKFSVRGEGEGDATEGKLTLKFICTTGKLPVPWPTLVTTLTYGVQCFSRYPDHMKRHDFFKSAMPEGYVQERTIEFKDDGTYKTRAEVKFEGDTLVNRIELKGNDFKEDGNILGHKLEYNHNSHNVRIEADKQKNGIKANFKIRHNVEDGSQQEADHKQQNTPIGDGPVRLPDNHYLSTQTTLSKDPNEKRDHMVLKEFVTAAGITKGEDERDKA

SEQ ID NO: 196 - protein, 222 aa, Artificial Sequence
  fusion protein
MEIYENENDQVEAVKRFFAENGKALAVGVILGVGALIGWRYWNSHQVDSARSASLAYQNAVTAVSEGKPDSIPAAEKFAAENKNTYGALASLELAQQFVDKNELEKAAAQLQQGLADTSDENLKAVINLRLARVQVQLKQADAALKTLDTIKGEGWAAIVADLRGEALLSKGDKQGARSAWEAGVKSDVTPALSEMMQMKINNLSIGSPSRLEEELRRRLTE

SEQ ID NO: 197 - protein, 222 aa, Artificial Sequence
  fusion protein
MEIYENENDQVEAVKRFFAENGKALAVGVILGVGALIGWRYWNSHQVDSARSASLAYQNAVTAVSEGKPDSIPAAEKFAAENKNTYGALASLELAQQFVDKNELEKAAAQLQQGLADTSDENLKAVINLRLARVQVQLKQADAALKTLDTIKGEGWAAIVADLRGEALLSKGDKQGARSAWEAGVKSDVTPALSEMMQMKINNLSIGSMSGRLEEELRRRLS

SEQ ID NO: 198 - protein, 206 aa, Artificial Sequence
  YfgM
MEIYENENDQVEAVKRFFAENGKALAVGVILGVGALIGWRYWNSHQVDSARSASLAYQNAVTAVSEGKPDSIPAAEKFAAENKNTYGALASLELAQQFVDKNELEKAAAQLQQGLADTSDENLKAVINLRLARVQVQLKQADAALKTLDTIKGEGWAAIVADLRGEALLSKGDKQGARSAWEAGVKSDVTPALSEMMQMKINNLSI

SEQ ID NO: 199 - protein, 260 aa, Artificial Sequence
  fusion protein
MSKHHHHSNHHRHNHHHHSGNHHHSGSAAGGEEDKKPAGGEGGGAHINLKVKGQDGNEVFFRIKRSTQLKKLMNAYCDRQSVDMTAIAFLFDGRRLRAEQTPDELEMEDGDEIDAMLHQTGGACAWSHPQFEKGGGSGGSSGGSAWSHPQFEKGSGSAESEAASSTMIKVKTLTGKEIEIDIEPTDTIDRIKERVEEKEGIPPVQQRLIYAGKQLADDKTAKDYNIEGGSVLHLVLALRGGATGTASTRLEEELRRRLAS